European Patent Application EP 4 285 913 A1, published December 6, 2023. Title: Highly Effective Adoptive T Cell Therapy. Applicant: ECOLE POLYTECHNIQUE FEDERALE DE LAUSANNE (EPFL). The sequence listing filed with the application follows.

SEQUENCE LISTING (22 sequences)

SEQ ID NO: 1 - protein, 129 aa, Homo sapiens [sequence omitted]

SEQ ID NO: 2 - protein, 232 aa, Homo sapiens
EPKSADKTHTCPPCPAPEAAGGPSVFLFPPKPKDTLMISRTPEVTCVVVDVSHEDPEVKFNWYVDGVEVHNAKTKPREEQYNSTYRVVSVLTVLHQDWLNGKEYKCKVSNKALGAPIEKTISKAKGQPREPQVYTLPPSREEMTKNQVSLTCLVKGFYPSDIAVEWESNGQPENNYKTTPPVLDSDGSFFLYSKLTVDKSRWQQGNVFSCSVMHEALHNHYTQKSLSLSPGK

SEQ ID NO: 3 - protein, 361 aa, Unknown
  synthetic peptide
HKCDITLQEIIKTLNSLTEQKTLCTELTVTDIFAASKNTTEKETFCRAATVLRQFYSHHEKDTRCLGATAQQFHRHKQLIRFLKRLDRNLWGLAGLNSCPVKEANQSTLENFLERLKTIMREKYSKCSSEPKSADKTHTCPPCPAPEAAGGPSVFLFPPKPKDTLMISRTPEVTCVVVDVSHEDPEVKFNWYVDGVEVHNAKTKPREEQYNSTYRVVSVLTVLHQDWLNGKEYKCKVSNKALGAPIEKTISKAKGQPREPQVYTLPPSREEMTKNQVSLTCLVKGFYPSDIAVEWESNGQPENNYKTTPPVLDSDGSFFLYSKLTVDKSRWQQGNVFSCSVMHEALHNHYTQKSLSLSPGK

SEQ ID NO: 4 - protein, 21 aa, Unknown
  synthetic peptide
GGSGGSGGSGGSGGSGGSGGS

SEQ ID NO: 5 - protein, 20 aa, Unknown
  synthetic peptide
GGGGSGGGGSGGGGSGGGGS

SEQ ID NO: 6 - protein, 382 aa, Unknown
  synthetic peptide
EPKSADKTHTCPPCPAPEAAGGPSVFLFPPKPKDTLMISRTPEVTCVVVDVSHEDPEVKFNWYVDGVEVHNAKTKPREEQYNSTYRVVSVLTVLHQDWLNGKEYKCKVSNKALGAPIEKTISKAKGQPREPQVYTLPPSREEMTKNQVSLTCLVKGFYPSDIAVEWESNGQPENNYKTTPPVLDSDGSFFLYSKLTVDKSRWQQGNVFSCSVMHEALHNHYTQKSLSLSPGKGGSGGSGGSGGSGGSGGSGGSHKCDITLQEIIKTLNSLTEQKTLCTELTVTDIFAASKNTTEKETFCRAATVLRQFYSHHEKDTRCLGATAQQFHRHKQLIRFLKRLDRNLWGLAGLNSCPVKEANQSTLENFLERLKTIMREKYSKCSS

SEQ ID NO: 7 - protein, 381 aa, Unknown
  synthetic peptide
EPKSADKTHTCPPCPAPEAAGGPSVFLFPPKPKDTLMISRTPEVTCVVVDVSHEDPEVKFNWYVDGVEVHNAKTKPREEQYNSTYRVVSVLTVLHQDWLNGKEYKCKVSNKALGAPIEKTISKAKGQPREPQVYTLPPSREEMTKNQVSLTCLVKGFYPSDIAVEWESNGQPENNYKTTPPVLDSDGSFFLYSKLTVDKSRWQQGNVFSCSVMHEALHNHYTQKSLSLSPGKGGGGSGGGGSGGGGSGGGGSHKCDITLQEIIKTLNSLTEQKTLCTELTVTDIFAASKNTTEKETFCRAATVLRQFYSHHEKDTRCLGATAQQFHRHKQLIRFLKRLDRNLWGLAGLNSCPVKEANQSTLENFLERLKTIMREKYSKCSS

SEQ ID NO: 8 - protein, 228 aa, Homo sapiens
ERKCCVECPPCPAPPVAGPSVFLFPPKPKDTLMISRTPEVTCVVVDVSHEDPEVQFNWYVDGVEVHNAKTKPREEQFNSTFRVVSVLTVVHQDWLNGKEYKCKVSNKGLPSSIEKTISKTKGQPREPQVYTLPPSREEMTKNQVSLTCLVKGFYPSDIAVEWESNGQPENNYKTTPPMLDSDGSFFLYSKLTVDKSRWQQGNVFSCSVMHEALHNHYTQKSLSLSPGK

SEQ ID NO: 9 - protein, 295 aa, Unknown
  synthetic peptide
TRCLGATAQQFHRHKQLIRFLKRLDRNLWGLAGLNSCPVKEANQSTLENFLERLKTIMREKYSKCSSERKCCVECPPCPAPPVAGPSVFLFPPKPKDTLMISRTPEVTCVVVDVSHEDPEVQFNWYVDGVEVHNAKTKPREEQFNSTFRVVSVLTVVHQDWLNGKEYKCKVSNKGLPSSIEKTISKTKGQPREPQVYTLPPSREEMTKNQVSLTCLVKGFYPSDIAVEWESNGQPENNYKTTPPMLDSDGSFFLYSKLTVDKSRWQQGNVFSCSVMHEALHNHYTQKSLSLSPGK

SEQ ID NO: 10 - protein, 378 aa, Unknown
  synthetic peptide
ERKCCVECPPCPAPPVAGPSVFLFPPKPKDTLMISRTPEVTCVVVDVSHEDPEVQFNWYVDGVEVHNAKTKPREEQFNSTFRVVSVLTVVHQDWLNGKEYKCKVSNKGLPSSIEKTISKTKGQPREPQVYTLPPSREEMTKNQVSLTCLVKGFYPSDIAVEWESNGQPENNYKTTPPMLDSDGSFFLYSKLTVDKSRWQQGNVFSCSVMHEALHNHYTQKSLSLSPGKGGSGGSGGSGGSGGSGGSGGSHKCDITLQEIIKTLNSLTEQKTLCTELTVTDIFAASKNTTEKETFCRAATVLRQFYSHHEKDTRCLGATAQQFHRHKQLIRFLKRLDRNLWGLAGLNSCPVKEANQSTLENFLERLKTIMREKYSKCSS

SEQ ID NO: 11 - protein, 279 aa, Homo sapiens
ELKTPLGDTTHTCPRCPEPKSCDTPPPCPRCPEPKSCDTPPPCPRCPEPKSCDTPPPCPRCPAPELLGGPSVFLFPPKPKDTLMISRTPEVTCVVVDVSHEDPEVQFKWYVDGVEVHNAKTKPREEQYNSTFRVVSVLTVLHQDWLNGKEYKCKVSNKALPAPIEKTISKTKGQPREPQVYTLPPSREEMTKNQVSLTCLVKGFYPSDIAVEWESSGQPENNYNTTPPMLDSDGSFFLYSKLTVDKSRWQQGNIFSCSVMHEALHNRFTQKSLSLSPGK

SEQ ID NO: 12 - protein, 408 aa, Unknown
  synthetic peptide
HKCDITLQEIIKTLNSLTEQKTLCTELTVTDIFAASKNTTEKETFCRAATVLRQFYSHHEKDTRCLGATAQQFHRHKQLIRFLKRLDRNLWGLAGLNSCPVKEANQSTLENFLERLKTIMREKYSKCSSELKTPLGDTTHTCPRCPEPKSCDTPPPCPRCPEPKSCDTPPPCPRCPEPKSCDTPPPCPRCPAPELLGGPSVFLFPPKPKDTLMISRTPEVTCVVVDVSHEDPEVQFKWYVDGVEVHNAKTKPREEQYNSTFRVVSVLTVLHQDWLNGKEYKCKVSNKALPAPIEKTISKTKGQPREPQVYTLPPSREEMTKNQVSLTCLVKGFYPSDIAVEWESSGQPENNYNTTPPMLDSDGSFFLYSKLTVDKSRWQQGNIFSCSVMHEALHNRFTQKSLSLSPGK

SEQ ID NO: 13 - protein, 429 aa, Unknown
  synthetic peptide
ELKTPLGDTTHTCPRCPEPKSCDTPPPCPRCPEPKSCDTPPPCPRCPEPKSCDTPPPCPRCPAPELLGGPSVFLFPPKPKDTLMISRTPEVTCVVVDVSHEDPEVQFKWYVDGVEVHNAKTKPREEQYNSTFRVVSVLTVLHQDWLNGKEYKCKVSNKALPAPIEKTISKTKGQPREPQVYTLPPSREEMTKNQVSLTCLVKGFYPSDIAVEWESSGQPENNYNTTPPMLDSDGSFFLYSKLTVDKSRWQQGNIFSCSVMHEALHNRFTQKSLSLSPGKGGSGGSGGSGGSGGSGGSGGSHKCDITLQEIIKTLNSLTEQKTLCTELTVTDIFAASKNTTEKETFCRAATVLRQFYSHHEKDTRCLGATAQQFHRHKQLIRFLKRLDRNLWGLAGLNSCPVKEANQSTLENFLERLKTIMREKYSKCSS

SEQ ID NO: 14 - protein, 229 aa, Homo sapiens
ESKYGPPCPPCPAPEFEGGPSVFLFPPKPKDTLMISRTPEVTCVVVDVSQEDPEVQFNWYVDGVEVHNAKTKPREEQFNSTYRVVSVLTVLHQDWLNGKEYKCKVSNKGLPSSIEKTISKAKGQPREPQVYTLPPSQEEMTKNQVSLTCLVKGFYPSDIAVEWESNGQPENNYKTTPPVLDSDGSFFLYSRLTVDKSRWQEGNVFSCSVMHEALHNHYTQKSLSLSLGK

SEQ ID NO: 15 - protein, 358 aa, Unknown
  synthetic peptide
HKCDITLQEIIKTLNSLTEQKTLCTELTVTDIFAASKNTTEKETFCRAATVLRQFYSHHEKDTRCLGATAQQFHRHKQLIRFLKRLDRNLWGLAGLNSCPVKEANQSTLENFLERLKTIMREKYSKCSSESKYGPPCPPCPAPEFEGGPSVFLFPPKPKDTLMISRTPEVTCVVVDVSQEDPEVQFNWYVDGVEVHNAKTKPREEQFNSTYRVVSVLTVLHQDWLNGKEYKCKVSNKGLPSSIEKTISKAKGQPREPQVYTLPPSQEEMTKNQVSLTCLVKGFYPSDIAVEWESNGQPENNYKTTPPVLDSDGSFFLYSRLTVDKSRWQEGNVFSCSVMHEALHNHYTQKSLSLSLGK

SEQ ID NO: 16 - protein, 379 aa, Unknown
  synthetic peptide
ESKYGPPCPPCPAPEFEGGPSVFLFPPKPKDTLMISRTPEVTCVVVDVSQEDPEVQFNWYVDGVEVHNAKTKPREEQFNSTYRVVSVLTVLHQDWLNGKEYKCKVSNKGLPSSIEKTISKAKGQPREPQVYTLPPSQEEMTKNQVSLTCLVKGFYPSDIAVEWESNGQPENNYKTTPPVLDSDGSFFLYSRLTVDKSRWQEGNVFSCSVMHEALHNHYTQKSLSLSLGKGGSGGSGGSGGSGGSGGSGGSHKCDITLQEIIKTLNSLTEQKTLCTELTVTDIFAASKNTTEKETFCRAATVLRQFYSHHEKDTRCLGATAQQFHRHKQLIRFLKRLDRNLWGLAGLNSCPVKEANQSTLENFLERLKTIMREKYSKCSS

SEQ ID NO: 17 - protein, 585 aa, Homo sapiens [sequence omitted]

SEQ ID NO: 18 - protein, 735 aa, Unknown
  synthetic peptide
HKCDITLQEIIKTLNSLTEQKTLCTELTVTDIFAASKNTTEKETFCRAATVLRQFYSHHEKDTRCLGATAQQFHRHKQLIRFLKRLDRNLWGLAGLNSCPVKEANQSTLENFLERLKTIMREKYSKCSSGGSGGSGGSGGSGGSGGSGGSDAHKSEVAHRFKDLGEENFKALVLIAFAQYLQQCPFEDHVKLVNEVTEFAKTCVADESAENCDKSLHTLFGDKLCTVATLRETYGEMADCCAKQEPERNECFLQHKDDNPNLPRLVRPEVDVMCTAFHDNEETFLKKYLYEIARRHPYFYAPELLFFAKRYKAAFTECCQAADKAACLLPKLDELRDEGKASSAKQRLKCASLQKFGERAFKAWAVARLSQRFPKAEFAEVSKLVTDLTKVHTECCHGDLLECADDRADLAKYICENQDSISSKLKECCEKPLLEKSHCIAEVENDEMPADLPSLAADFVESKDVCKNYAEAKDVFLGMFLYEYARRHPDYSVVLLLRLAKTYETTLEKCCAAADPHECYAKVFDEFKPLVEEPQNLIKQNCELFEQLGEYKFQNALLVRYTKKVPQVSTPTLVEVSRNLGKVGSKCCKHPEAKRMPCAEDYLSVVLNQLCVLHEKTPVSDRVTKCCTESLVNRRPCFSALEVDETYVPKEFNAETFTFHADICTLSEKERQIKKQTALVELVKHKPKATKEQLKAVMDDFAAFVEKCCKADDKETCFAEEGKKLVAASQAALGL

SEQ ID NO: 19 - protein, 735 aa, Unknown
  synthetic ppetide
DAHKSEVAHRFKDLGEENFKALVLIAFAQYLQQCPFEDHVKLVNEVTEFAKTCVADESAENCDKSLHTLFGDKLCTVATLRETYGEMADCCAKQEPERNECFLQHKDDNPNLPRLVRPEVDVMCTAFHDNEETFLKKYLYEIARRHPYFYAPELLFFAKRYKAAFTECCQAADKAACLLPKLDELRDEGKASSAKQRLKCASLQKFGERAFKAWAVARLSQRFPKAEFAEVSKLVTDLTKVHTECCHGDLLECADDRADLAKYICENQDSISSKLKECCEKPLLEKSHCIAEVENDEMPADLPSLAADFVESKDVCKNYAEAKDVFLGMFLYEYARRHPDYSVVLLLRLAKTYETTLEKCCAAADPHECYAKVFDEFKPLVEEPQNLIKQNCELFEQLGEYKFQNALLVRYTKKVPQVSTPTLVEVSRNLGKVGSKCCKHPEAKRMPCAEDYLSVVLNQLCVLHEKTPVSDRVTKCCTESLVNRRPCFSALEVDETYVPKEFNAETFTFHADICTLSEKERQIKKQTALVELVKHKPKATKEQLKAVMDDFAAFVEKCCKADDKETCFAEEGKKLVAASQAALGLGGSGGSGGSGGSGGSGGSGGSHKCDITLQEIIKTLNSLTEQKTLCTELTVTDIFAASKNTTEKETFCRAATVLRQFYSHHEKDTRCLGATAQQFHRHKQLIRFLKRLDRNLWGLAGLNSCPVKEANQSTLENFLERLKTIMREKYSKCSS

SEQ ID NO: 20 - protein, 120 aa, Mus musculus
HIHGCDKNHLREIIGILNEVTGEGTPCTEMDVPNVLTATKNTTESELVCRASKVLRIFYLKHGKTPCLKKNSSVLMELQRLFRAFRCLDSSISCTMNESKSTSLKDFLESLKSIMQMDYS

SEQ ID NO: 21 - protein, 238 aa, Mus musculus
EPRVPITQNPCPPLKECPPCAAPDLLGGPSVFIFPPKIKDVLMISLSPMVTCVVVAVSEDDPDVQISWFVNNVEVHTAQTQTHREDYNSTLRVVSALPIQHQDWMSGKEFKCKVNNRALPSPIEKTISKPRGPVRAPQVYVLPPPAEEMTKKEFSLTCMITGFLPAEIAVDWTSNGRTEQNYKNTATVLDSDGSYFMYSKLRVQKSTWERGSLFACSVVHEGLHNHLTTKTISRSLGK

SEQ ID NO: 22 - protein, 379 aa, Mus musculus
EPRVPITQNPCPPLKECPPCAAPDLLGGPSVFIFPPKIKDVLMISLSPMVTCVVVAVSEDDPDVQISWFVNNVEVHTAQTQTHREDYNSTLRVVSALPIQHQDWMSGKEFKCKVNNRALPSPIEKTISKPRGPVRAPQVYVLPPPAEEMTKKEFSLTCMITGFLPAEIAVDWTSNGRTEQNYKNTATVLDSDGSYFMYSKLRVQKSTWERGSLFACSVVHEGLHNHLTTKTISRSLGKGGSGGSGGSGGSGGSGGSGGSHIHGCDKNHLREIIGILNEVTGEGTPCTEMDVPNVLTATKNTTESELVCRASKVLRIFYLKHGKTPCLKKNSSVLMELQRLFRAFRCLDSSISCTMNESKSTSLKDFLESLKSIMQMDYS